European Patent Specification EP 3 484 922 B1, published April 29, 2026. Title: MULTISPECIFIC ANTIBODIES AGAINST CD40 AND CD137. Applicant: Genmab A/S. The sequence listing filed with the application follows.

SEQUENCE LISTING (136 sequences)

SEQ ID NO: 1 - protein, 8 aa, Mus Musculus
GYTFTEYI

SEQ ID NO: 2 - protein, 8 aa, Mus Musculus
IIPNNGGT

SEQ ID NO: 3 - protein, 15 aa, Mus Musculus
TRREVYGRNYYALDY

SEQ ID NO: 4 - protein, 6 aa, Mus Musculus
QGINNY

SEQ ID NO: 5 - protein, 9 aa, Mus Musculus
QQYSNLPYT

SEQ ID NO: 6 - protein, 122 aa, Mus Musculus
EVQLQQSGPDLVKPGASVKISCKTSGYTFTEYIMHWVKQSHGKSLEWIGGIIPNNGGTSYNQKFKDKATMTVDKSSSTGYMELRSLTSEDSAVYYCTRREVYGRNYYALDYWGQGTLVTVSS

SEQ ID NO: 7 - protein, 107 aa, Mus Musculus
DIQMTQTTSSLSASLGDRVTITCSASQGINNYLNWYQQKPDGTVKLLIYYTSSLHSGVPSRFSGSGSGTDYSLTISNLEPEDIATYYCQQYSNLPYTFGGGTKLEIK

SEQ ID NO: 8 - protein, 8 aa, Oryctolagus cuniculus
GFSLSSYA

SEQ ID NO: 9 - protein, 7 aa, Oryctolagus cuniculus
IWNNGAT

SEQ ID NO: 10 - protein, 14 aa, Oryctolagus cuniculus
ARSANDAWSTYSDL

SEQ ID NO: 11 - protein, 6 aa, Oryctolagus cuniculus
QTITNY

SEQ ID NO: 12 - protein, 14 aa, Oryctolagus cuniculus
QNYYYGSSSGYGFV

SEQ ID NO: 13 - protein, 117 aa, Oryctolagus cuniculus
QSVEESGGRLVTPGTPLTLTCTVSGFSLSSYAVSWVRQAPGKGLEWIGVIWNNGATHYATWAKGRFTISKASTTVDLKVTSPTTEDTATYFCARSANDAWSTYSDLWGQGTLVTVSS

SEQ ID NO: 14 - protein, 112 aa, Oryctolagus cuniculus
DIVMTQTPASVEAAVGGTVTIKCQASQTITNYLSWYQQKPGQPPKLLIYKASTLTSGVSSRFKGSGSGTEFTLTISDLESDDAATYYCQNYYYGSSSGYGFVFGGGTEVVVK

SEQ ID NO: 15 - protein, 8 aa, Oryctolagus cuniculus
GFSLTYYA

SEQ ID NO: 16 - protein, 7 aa, Oryctolagus cuniculus
IYDNGAT

SEQ ID NO: 17 - protein, 14 aa, Oryctolagus cuniculus
ARSANNAWSTYSNL

SEQ ID NO: 18 - protein, 6 aa, Oryctolagus cuniculus
EDISSY

SEQ ID NO: 19 - protein, 14 aa, Oryctolagus cuniculus
QSYYSGSISGYGFV

SEQ ID NO: 20 - protein, 117 aa, Oryctolagus cuniculus
QSVEESGGRLVTPGTPLTLTCTVSGFSLTYYAVTWVRQPPGKGLEWIGVIYDNGATAFATWAKGRFTMSKNSTTVALKVTSPTTEDTATYFCARSANNAWSTYSNLWGQGTLVTVSS

SEQ ID NO: 21 - protein, 112 aa, Oryctolagus cuniculus
DIVMTQTPSSVSAAVGGTVTINCQASEDISSYLSWYQQKLGQPPKLLIYKASTLESGVPSRFKGSGSGTEYTLTISDLESDDAATYYCQSYYSGSISGYGFVFGGGTGVVVK

SEQ ID NO: 22 - protein, 8 aa, Oryctolagus cuniculus
GFTISSYH

SEQ ID NO: 23 - protein, 8 aa, Oryctolagus cuniculus
IYGGTATT

SEQ ID NO: 24 - protein, 17 aa, Oryctolagus cuniculus
ARARYSGGSYANYVFNL

SEQ ID NO: 25 - protein, 6 aa, Oryctolagus cuniculus
QSISSY

SEQ ID NO: 26 - protein, 14 aa, Oryctolagus cuniculus
QGYDWSSSNRYDNT

SEQ ID NO: 27 - protein, 121 aa, Oryctolagus cuniculus
QSVEESGGRLVTPGTPLTLTCTASGFTISSYHMIWVRQAPGEGLEWIGDIYGGTATTDYASWAKGRFTISKTSTTVDLKMTSLTTEDTATYFCARARYSGGSYANYVFNLWGQGTLVTVSS

SEQ ID NO: 28 - protein, 112 aa, Oryctolagus cuniculus
DIVMTQTPASVEAAVGGTVTIKCQASQSISSYLAWYQQKPGQPPKLLIYRTSTLESGVPSRFKGSGSGTEFTLTISDLESADAATYYCQGYDWSSSNRYDNTFGGGTEVVVK

SEQ ID NO: 29 - protein, 8 aa, Oryctolagus cuniculus
GFSLSRYD

SEQ ID NO: 30 - protein, 7 aa, Oryctolagus cuniculus
ISSSGGT

SEQ ID NO: 31 - protein, 11 aa, Oryctolagus cuniculus
AREGDYWDFNL

SEQ ID NO: 32 - protein, 6 aa, Oryctolagus cuniculus
QSISNL

SEQ ID NO: 33 - protein, 12 aa, Oryctolagus cuniculus
AGGFPGLDTVAA

SEQ ID NO: 34 - protein, 114 aa, Oryctolagus cuniculus
QSLEESGGRLVTPGTPLTLTCTASGFSLSRYDMSWVRQAPGKGLEYIGVISSSGGTNYANWAKGRFTISKTSTTVDLKITSPTTEDTATYFCAREGDYWDFNLWGPGTLVTVSS

SEQ ID NO: 35 - protein, 110 aa, Oryctolagus cuniculus
AQVLTQTPSSVSAAVGGTVTINCQASQSISNLLAWYQQKPGQPPKLLIYGASTLASGVPSRFSGSGSGTEFTLTISDLESDDAATYYCAGGFPGLDTVAAFGGGTEAVVT

SEQ ID NO: 36 - protein, 8 aa, Oryctolagus cuniculus
GFTISDFH

SEQ ID NO: 37 - protein, 8 aa, Oryctolagus cuniculus
IITSASTT

SEQ ID NO: 38 - protein, 15 aa, Oryctolagus cuniculus
ARSTYTDTSGYYFDF

SEQ ID NO: 39 - protein, 8 aa, Oryctolagus cuniculus
QSIYNGNR

SEQ ID NO: 40 - protein, 13 aa, Oryctolagus cuniculus
LGSYDCDSADCFA

SEQ ID NO: 41 - protein, 119 aa, Oryctolagus cuniculus
QSVEESGGRLVTPGTPLTLTCTASGFTISDFHVTWVRQAPGKGLEWIGTIITSASTTAYATWARGRFTISKSSTTVNLKIVSPTTEDTATYFCARSTYTDTSGYYFDFWGQGTLVTVSS

SEQ ID NO: 42 - protein, 113 aa, Oryctolagus cuniculus
AQVLTQTASPVSAAVGGTVIINCQSSQSIYNGNRLSWYQQKPGQPPKLLIYSASTLASGVSSRFKGSGSGTQFTLAISDVQSDDAATYYCLGSYDCDSADCFAFGGGTEVVVE

SEQ ID NO: 43 - protein, 8 aa, Oryctolagus cuniculus
GFSLSSYA

SEQ ID NO: 44 - protein, 7 aa, Oryctolagus cuniculus
ISTSGIT

SEQ ID NO: 45 - protein, 15 aa, Oryctolagus cuniculus
ARLNGFDDYVRYFDF

SEQ ID NO: 46 - protein, 6 aa, Oryctolagus cuniculus
ESIASN

SEQ ID NO: 47 - protein, 12 aa, Oryctolagus cuniculus
QSAFYVSSSDNA

SEQ ID NO: 48 - protein, 118 aa, Oryctolagus cuniculus
QSVEESGGRLVTPGTPLTLTCTVSGFSLSSYAMSWVRQAPGKGLEWIGIISTSGITYYASWAKGRFTISKTSTMVDLKITSPTTEDTATYFCARLNGFDDYVRYFDFWGLGTLVTVSS

SEQ ID NO: 49 - protein, 110 aa, Oryctolagus cuniculus
AIELTQTPSSVSAAVGGTVTINCQASESIASNLAWYQQKPGQPPKLLIYAASYLASGVPSRFKGSGSGTEYTLTISGVQSADAATYYCQSAFYVSSSDNAFGGGTEVVVK

SEQ ID NO: 50 - protein, 8 aa, Oryctolagus cuniculus
GFSLSSYD

SEQ ID NO: 51 - protein, 7 aa, Oryctolagus cuniculus
IGSDGSA

SEQ ID NO: 52 - protein, 12 aa, Oryctolagus cuniculus
ARDWNDYWAHDL

SEQ ID NO: 53 - protein, 8 aa, Oryctolagus cuniculus
QIVTSKSA

SEQ ID NO: 54 - protein, 12 aa, Oryctolagus cuniculus
AGGYYNSGDLNP

SEQ ID NO: 55 - protein, 115 aa, Oryctolagus cuniculus
QSLEESGGRLVTPGTPLTLTCTASGFSLSSYDVSWVRQAPGKGLEYIGFIGSDGSAHYATWVKGRFTISKTSTTVDLKITSPTTEDTATYFCARDWNDYWAHDLWGPGTLVTVSS

SEQ ID NO: 56 - protein, 112 aa, Oryctolagus cuniculus
AQVLTQTTSPVSAAVGGTVTINCQASQIVTSKSALSWYQQKPGQPPRLLIYKASTLASGVPSRFSGSGSGTQFTLTISDLESDDAATYYCAGGYYNSGDLNPFGGGTEVVVK

SEQ ID NO: 57 - protein, 8 aa, Oryctolagus cuniculus
GFSLSSYD

SEQ ID NO: 58 - protein, 7 aa, Oryctolagus cuniculus
ISSSGNT

SEQ ID NO: 59 - protein, 11 aa, Oryctolagus cuniculus
AREGDYWDFNL

SEQ ID NO: 60 - protein, 6 aa, Oryctolagus cuniculus
QSISNL

SEQ ID NO: 61 - protein, 12 aa, Oryctolagus cuniculus
AGGFPGLDTGAT

SEQ ID NO: 62 - protein, 114 aa, Oryctolagus cuniculus
QSLEESGGRLVTPGTPLTLTCTASGFSLSSYDMSWVRQAPGKGLEYIGYISSSGNTYYASWAKSRFTISKTSTTVDLKITSPTTEDTATYFCAREGDYWDFNLWGPGTLVTVSS

SEQ ID NO: 63 - protein, 110 aa, Oryctolagus cuniculus
AQVLTQTPSSVSAAVGGTVTINCQASQSISNLLAWYQQKPGQRPRLLIYRASTLASGVPSRFKGSGSGTEFTLTISDLESEDAATYYCAGGFPGLDTGATFGGGTEAVVT

SEQ ID NO: 64 - protein, 8 aa, Oryctolagus cuniculus
GFSLNDYW

SEQ ID NO: 65 - protein, 7 aa, Oryctolagus cuniculus
IDVGGSL

SEQ ID NO: 66 - protein, 11 aa, Oryctolagus cuniculus
ARGGLTYGFDL

SEQ ID NO: 67 - protein, 6 aa, Oryctolagus cuniculus
EDISSY

SEQ ID NO: 68 - protein, 12 aa, Oryctolagus cuniculus
HYYATISGLGVA

SEQ ID NO: 69 - protein, 114 aa, Oryctolagus cuniculus
QSLEESGGRLVTPGTPLTLTCTVSGFSLNDYWMSWVRQAPGKGLEWIGYIDVGGSLYYASWAKGRFTISRTSTTVDLKMTSLTTEDTATYFCARGGLTYGFDLWGPGTLVTVSS

SEQ ID NO: 70 - protein, 110 aa, Oryctolagus cuniculus
DIVMTQTPASVSEPVGGTVTINCQASEDISSYLAWYQQKPGQRPKRLIYGASDLASGVPSRFSASGSGTEYALTISDLESADAATYYCHYYATISGLGVAFGGGTEVVVK

SEQ ID NO: 71 - protein, 8 aa, Oryctolagus cuniculus
GFSLSTYA

SEQ ID NO: 72 - protein, 7 aa, Oryctolagus cuniculus
VYDNGYI

SEQ ID NO: 73 - protein, 14 aa, Oryctolagus cuniculus
ARSADGSWSTYFNL

SEQ ID NO: 74 - protein, 6 aa, Oryctolagus cuniculus
ESISNY

SEQ ID NO: 75 - protein, 14 aa, Oryctolagus cuniculus
QTNYCCSSSDNGFA

SEQ ID NO: 76 - protein, 117 aa, Oryctolagus cuniculus
QSVEESGGRLVTPGTPLTLTCTVSGFSLSTYAMIWVRQAPGKGLEWIGVVYDNGYISHATWVKGRFTISKTSTTVGLEITSPTTEDTATYFCARSADGSWSTYFNLWGQGTLVTVSS

SEQ ID NO: 77 - protein, 112 aa, Oryctolagus cuniculus
DIVMTQTPASVEAAVGGTVTIKCQASESISNYLAWYQQKPGQPPKLLIYKASTLASGVSSRFKGSGSGTEFTLTISDLESADAATYYCQTNYCCSSSDNGFAFGGGTEVVVK

SEQ ID NO: 78 - protein, 8 aa, Oryctolagus cuniculus
GIDLSSYH

SEQ ID NO: 79 - protein, 7 aa, Oryctolagus cuniculus
IAYGGNT

SEQ ID NO: 80 - protein, 12 aa, Oryctolagus cuniculus
ARGYSEDSYWGL

SEQ ID NO: 81 - protein, 6 aa, Oryctolagus cuniculus
QNIENY

SEQ ID NO: 82 - protein, 12 aa, Oryctolagus cuniculus
QQDYGIIFVDNI

SEQ ID NO: 83 - protein, 115 aa, Oryctolagus cuniculus
QSLEESGGRLVTPGTPLTLTCTVSGIDLSSYHMCWVRQAPGKGLEYIGYIAYGGNTYYANWAKGRFTISKTSTTVDLRITSPTTEDTATYFCARGYSEDSYWGLWGPGTLVTVSS

SEQ ID NO: 84 - protein, 110 aa, Oryctolagus cuniculus
AYDMTQTPASVEAAVGGTVTIKCQASQNIENYLAWYQQKPGQPPKLLIYDTSKLTSGVPSRFSGSGSGTDFTLTISGVQSDDAATYYCQQDYGIIFVDNIFGGGTEVVVK

SEQ ID NO: 85 - protein, 8 aa, Oryctolagus cuniculus
GFSLSDYY

SEQ ID NO: 86 - protein, 7 aa, Oryctolagus cuniculus
MSGSGST

SEQ ID NO: 87 - protein, 18 aa, Oryctolagus cuniculus
ARDGDYAGWGYATGAFDP

SEQ ID NO: 88 - protein, 8 aa, Oryctolagus cuniculus
QSVVGNSL

SEQ ID NO: 89 - protein, 12 aa, Oryctolagus cuniculus
TGRYNSDTDTFV

SEQ ID NO: 90 - protein, 122 aa, Oryctolagus cuniculus
QSVEESGGRLVTPGTPLTLTCTVSGFSLSDYYMTWVRQAPGKGLEYIGIMSGSGSTYYASWAKGRFTISKTSSTTLELKITSPTTEDTAIYFCARDGDYAGWGYATGAFDPWGPGTLVTVSS

SEQ ID NO: 91 - protein, 112 aa, Oryctolagus cuniculus
AAVLTQTPSPVSAAVGGTVTISCQASQSVVGNSLLSWFQKKPGQPPKLLIYSASSLASGVPSRFKGSGSGTQFTLTISDLESDDAATYYCTGRYNSDTDTFVFGGGTEVVVK

SEQ ID NO: 92 - protein, 255 aa, homo sapiens
MGNSCYNIVATLLLVLNFERTRSLQDPCSNCPAGTFCDNNRNQICSPCPPNSFSSAGGQRTCDICRQCKGVFRTRKECSSTSNAECDCTPGFHCLGAGCSMCEQDCKQGQELTKKGCKDCCFGTFNDQKRGICRPWTNCSLDGKSVLVNGTKERDVVCGPSPADLSPGASSVTPPAPAREPGHSPQIISFFLALTSTALLFLLFFLTLRFSVVKRGRKKLLYIFKQPFMRPVQTTQEEDGCSCRFPEEEEGGCEL

SEQ ID NO: 93 - protein, 205 aa, artificial sequence
  N/A
MGNSCYNIVATLLLVLNFERTRSVPDPCSNCSAGTFCGKNIQELCMPCPPNSFSSAGGQRTCDICRQCKGVFRTRKECSSTSNAECDCTPGFHCLGAGCSMCEQDCKQGQELTKKGCKDCCFGTFNDQKRGICRPWTNCSLDGKSVLVNGTKERDVVCGPSPADLSPGASSVTPPAPAREPGHSPQIISFFLALTSTALLGGCEL

SEQ ID NO: 94 - protein, 255 aa, artificial sequence
  N/A
MGNSCYNIVATLLLVLNFERTRSLQDPCSNCPAGTFCDNNRNQICSPCPLNSFSSTGGQMNCDMCRKCEGVFKTKRACSPTRDAECECTPGFHCLGAGCSMCEQDCKQGQELTKKGCKDCCFGTFNDQKRGICRPWTNCSLDGKSVLVNGTKERDVVCGPSPADLSPGASSVTPPAPAREPGHSPQIISFFLALTSTALLFLLFFLTLRFSVVKRGRKKLLYIFKQPFMRPVQTTQEEDGCSCRFPEEEEGGCEL

SEQ ID NO: 95 - protein, 255 aa, artificial sequence
  N/A
MGNSCYNIVATLLLVLNFERTRSLQDPCSNCPAGTFCDNNRNQICSPCPPNSFSSAGGQRTCDICRQCKGVFRTRKECSSTSNAECDCVPGFRCLGAGCAMCEEYCQQGQELTQKGCKDCCFGTFNDQKRGICRPWTNCSLDGKSVLVNGTKERDVVCGPSPADLSPGASSVTPPAPAREPGHSPQIISFFLALTSTALLFLLFFLTLRFSVVKRGRKKLLYIFKQPFMRPVQTTQEEDGCSCRFPEEEEGGCEL

SEQ ID NO: 96 - protein, 255 aa, artificial sequence
  N/A
MGNSCYNIVATLLLVLNFERTRSLQDPCSNCPAGTFCDNNRNQICSPCPPNSFSSAGGQRTCDICRQCKGVFRTRKECSSTSNAECDCTPGFHCLGAGCSMCEQDCKQGQELTKEGCKDCSFGTFNDEEHGVCRPWTDCSLDGKSVLVNGTKERDVVCGPSPADLSPGASSVTPPAPAREPGHSPQIISFFLALTSTALLFLLFFLTLRFSVVKRGRKKLLYIFKQPFMRPVQTTQEEDGCSCRFPEEEEGGCEL

SEQ ID NO: 97 - protein, 255 aa, artificial sequence
  N/A
MGNSCYNIVATLLLVLNFERTRSLQDPCSNCPAGTFCDNNRNQICSPCPPNSFSSAGGQRTCDICRQCKGVFRTRKECSSTSNAECDCTPGFHCLGAGCSMCEQDCKQGQELTKKGCKDCCFGTFNDQKRGICRPWTNCSLAGKPVLMNGTKARDVVCGPRPADLSPGASSVTPPAPAREPGHSPQIISFFLALTSTALLFLLFFLTLRFSVVKRGRKKLLYIFKQPFMRPVQTTQEEDGCSCRFPEEEEGGCEL

SEQ ID NO: 98 - protein, 255 aa, artificial sequence
  N/A
MGNSCYNIVATLLLVLNFERTRSLQDPCSNCPAGTFCDNNRNQICSPCPPNSFSSAGGQRTCDICRQCKGVFRTRKECSSTSNAECDCTPGFHCLGAGCSMCEQDCKQGQELTKKGCKDCCFGTFNDQKRGICRPWTNCSLDGKSVLVNGTKERDVVCGPSPTDFSPGTPSTTMPVPGGEPGHTSHIISFFLALTSTALLFLLFFLTLRFSVVKRGRKKLLYIFKQPFMRPVQTTQEEDGCSCRFPEEEEGGCEL

SEQ ID NO: 99 - protein, 8 aa, homo sapiens
GYRFSNFV

SEQ ID NO: 100 - protein, 8 aa, homo sapiens
INPYNGNK

SEQ ID NO: 101 - protein, 20 aa, homo sapiens
ARVGPYSWDDSPQDNYYMDV

SEQ ID NO: 102 - protein, 7 aa, homo sapiens
HSIRSRR

SEQ ID NO: 103 - protein, 9 aa, homo sapiens
QVYGASSYT

SEQ ID NO: 104 - protein, 127 aa, homo sapiens
QVQLVQSGAEVKKPGASVKVSCQASGYRFSNFVIHWVRQAPGQRFEWMGWINPYNGNKEFSAKFQDRVTFTADTSANTAYMELRSLRSADTAVYYCARVGPYSWDDSPQDNYYMDVWGKGTTVIVSS

SEQ ID NO: 105 - protein, 108 aa, homo sapiens
EIVLTQSPGTLSLSPGERATFSCRSSHSIRSRRVAWYQHKPGQAPRLVIHGVSNRASGISDRFSGSGSGTDFTLTITRVEPEDFALYYCQVYGASSYTFGQGTKLERK

SEQ ID NO: 106 - protein, 107 aa, homo sapiens
GQPREPQVYTLPPSRDELTKNQVSLTCLVKGFYPSDIAVEWESNGQPENNYKTTPPVLDSDGSFFLYSKLTVDKSRWQQGNVFSCSVMHEALHNHYTQKSLSLSPGK

SEQ ID NO: 107 - protein, 107 aa, homo sapiens
GQPREPQVYTLPPSREEMTKNQVSLTCLVKGFYPSDIAVEWESNGQPENNYKTTPPVLDSDGSFFLYSKLTVDKSRWQQGNVFSCSVMHEALHNHYTQKSLSLSPGK

SEQ ID NO: 108 - protein, 107 aa, homo sapiens
GQPREPQVYTLPPSRDELTKNQVSLTCLVKGFYPSDIAVEWESNGQPENNYKTTPPVLDSDGSFFLYSKLTVDKSRWQQGNVFSCSVMHEGLHNHYTQKSLSLSPGK

SEQ ID NO: 109 - protein, 330 aa, homo sapiens
ASTKGPSVFPLAPSSKSTSGGTAALGCLVKDYFPEPVTVSWNSGALTSGVHTFPAVLQSSGLYSLSSVVTVPSSSLGTQTYICNVNHKPSNTKVDKRVEPKSCDKTHTCPPCPAPELLGGPSVFLFPPKPKDTLMISRTPEVTCVVVDVSHEDPEVKFNWYVDGVEVHNAKTKPREEQYNSTYRVVSVLTVLHQDWLNGKEYKCKVSNKALPAPIEKTISKAKGQPREPQVYTLPPSREEMTKNQVSLTCLVKGFYPSDIAVEWESNGQPENNYKTTPPVLDSDGSFFLYSKLTVDKSRWQQGNVFSCSVMHEALHNHYTQKSLSLSPGK

SEQ ID NO: 110 - protein, 330 aa, Artificial Sequence
  N/A
ASTKGPSVFPLAPSSKSTSGGTAALGCLVKDYFPEPVTVSWNSGALTSGVHTFPAVLQSSGLYSLSSVVTVPSSSLGTQTYICNVNHKPSNTKVDKRVEPKSCDKTHTCPPCPAPELLGGPSVFLFPPKPKDTLMISRTPEVTCVVVDVSHEDPEVKFNWYVDGVEVHNAKTKPREEQYNSTYRVVSVLTVLHQDWLNGKEYKCKVSNKALPAPIEKTISKAKGQPREPQVYTLPPSREEMTKNQVSLTCLVKGFYPSDIAVEWESNGQPENNYKTTPPVLDSDGSFLLYSKLTVDKSRWQQGNVFSCSVMHEALHNHYTQKSLSLSPGK

SEQ ID NO: 111 - protein, 330 aa, Artificial Sequence
  N/A
ASTKGPSVFPLAPSSKSTSGGTAALGCLVKDYFPEPVTVSWNSGALTSGVHTFPAVLQSSGLYSLSSVVTVPSSSLGTQTYICNVNHKPSNTKVDKRVEPKSCDKTHTCPPCPAPELLGGPSVFLFPPKPKDTLMISRTPEVTCVVVDVSHEDPEVKFNWYVDGVEVHNAKTKPREEQYNSTYRVVSVLTVLHQDWLNGKEYKCKVSNKALPAPIEKTISKAKGQPREPQVYTLPPSREEMTKNQVSLTCLVKGFYPSDIAVEWESNGQPENNYKTTPPVLDSDGSFFLYSRLTVDKSRWQQGNVFSCSVMHEALHNHYTQKSLSLSPGK

SEQ ID NO: 112 - protein, 330 aa, Artificial Sequence
  N/A
ASTKGPSVFPLAPSSKSTSGGTAALGCLVKDYFPEPVTVSWNSGALTSGVHTFPAVLQSSGLYSLSSVVTVPSSSLGTQTYICNVNHKPSNTKVDKRVEPKSCDKTHTCPPCPAPEFEGGPSVFLFPPKPKDTLMISRTPEVTCVVVAVSHEDPEVKFNWYVDGVEVHNAKTKPREEQYNSTYRVVSVLTVLHQDWLNGKEYKCKVSNKALPAPIEKTISKAKGQPREPQVYTLPPSREEMTKNQVSLTCLVKGFYPSDIAVEWESNGQPENNYKTTPPVLDSDGSFFLYSRLTVDKSRWQQGNVFSCSVMHEALHNHYTQKSLSLSPGK

SEQ ID NO: 113 - protein, 330 aa, Artificial Sequence
  N/A
ASTKGPSVFPLAPSSKSTSGGTAALGCLVKDYFPEPVTVSWNSGALTSGVHTFPAVLQSSGLYSLSSVVTVPSSSLGTQTYICNVNHKPSNTKVDKRVEPKSCDKTHTCPPCPAPEFEGGPSVFLFPPKPKDTLMISRTPEVTCVVVAVSHEDPEVKFNWYVDGVEVHNAKTKPREEQYNSTYRVVSVLTVLHQDWLNGKEYKCKVSNKALPAPIEKTISKAKGQPREPQVYTLPPSREEMTKNQVSLTCLVKGFYPSDIAVEWESNGQPENNYKTTPPVLDSDGSFLLYSKLTVDKSRWQQGNVFSCSVMHEALHNHYTQKSLSLSPGK

SEQ ID NO: 114 - protein, 107 aa, Homo Sapiens [sequence omitted]

SEQ ID NO: 115 - protein, 277 aa, Homo Sapiens
MVRLPLQCVLWGCLLTAVHPEPPTACREKQYLINSQCCSLCQPGQKLVSDCTEFTETECLPCGESEFLDTWNRETHCHQHKYCDPNLGLRVQQKGTSETDTICTCEEGWHCTSEACESCVLHRSCSPGFGVKQIATGVSDTICEPCPVGFFSNVSSAFEKCHPWTSCETKDLVVQQAGTNKTDVVCGPQDRLRALVVIPIIFGILFAILLVLVFIKKVAKKPTNKAPHPKQEPQEINFPDDLPGSNTAAPVQETLHGCQPVTQEDGKESRISVQERQ

SEQ ID NO: 116 - protein, 330 aa, Homo Sapiens
ASTKGPSVFPLAPSSKSTSGGTAALGCLVKDYFPEPVTVSWNSGALTSGVHTFPAVLQSSGLYSLSSVVTVPSSSLGTQTYICNVNHKPSNTKVDKRVEPKSCDKTHTCPPCPAPEFEGGPSVFLFPPKPKDTLMISRTPEVTCVVVAVSHEDPEVKFNWYVDGVEVHNAKTKPREEQYNSTYRVVSVLTVLHQDWLNGKEYKCKVSNKALPAPIEKTISKAKGQPREPQVYTLPPSREEMTKNQVSLTCLVKGFYPSDIAVEWESNGQPENNYKTTPPVLDSDGSFFLYSKLTVDKSRWQQGNVFSCSVMHEALHNHYTQKSLSLSPGK

SEQ ID NO: 117 - protein, 122 aa, Artificial Sequence
  N/A
EVQLVQSGAEVKKPGASVKVSCKTSGYTFTEYIMHWVRQAPGQGLEWMGGIIPNNGGTSYNQKFQGRVTMTVDKSTSTGYMELSSLRSEDTAVYYCTRREVYGRNYYALDYWGQGTLVTVSS

SEQ ID NO: 118 - protein, 452 aa, Artificial Sequence
  N/A
EVQLVQSGAEVKKPGASVKVSCKTSGYTFTEYIMHWVRQAPGQGLEWMGGIIPNNGGTSYNQKFQGRVTMTVDKSTSTGYMELSSLRSEDTAVYYCTRREVYGRNYYALDYWGQGTLVTVSSASTKGPSVFPLAPSSKSTSGGTAALGCLVKDYFPEPVTVSWNSGALTSGVHTFPAVLQSSGLYSLSSVVTVPSSSLGTQTYICNVNHKPSNTKVDKRVEPKSCDKTHTCPPCPAPELLGGPSVFLFPPKPKDTLMISRTPEVTCVVVDVSHEDPEVKFNWYVDGVEVHNAKTKPREEQYNSTYRVVSVLTVLHQDWLNGKEYKCKVSNKALPAPIEKTISKAKGQPREPQVYTLPPSREEMTKNQVSLTCLVKGFYPSDIAVEWESNGQPENNYKTTPPVLDSDGSFFLYSKLTVDKSRWQQGNVFSCSVMHEALHNHYTQKSLSLSPGK

SEQ ID NO: 119 - protein, 452 aa, Artificial Sequence
  N/A
EVQLVQSGAEVKKPGASVKVSCKTSGYTFTEYIMHWVRQAPGQGLEWMGGIIPNNGGTSYNQKFQGRVTMTVDKSTSTGYMELSSLRSEDTAVYYCTRREVYGRNYYALDYWGQGTLVTVSSASTKGPSVFPLAPSSKSTSGGTAALGCLVKDYFPEPVTVSWNSGALTSGVHTFPAVLQSSGLYSLSSVVTVPSSSLGTQTYICNVNHKPSNTKVDKRVEPKSCDKTHTCPPCPAPEFEGGPSVFLFPPKPKDTLMISRTPEVTCVVVAVSHEDPEVKFNWYVDGVEVHNAKTKPREEQYNSTYRVVSVLTVLHQDWLNGKEYKCKVSNKALPAPIEKTISKAKGQPREPQVYTLPPSREEMTKNQVSLTCLVKGFYPSDIAVEWESNGQPENNYKTTPPVLDSDGSFLLYSKLTVDKSRWQQGNVFSCSVMHEALHNHYTQKSLSLSPGK

SEQ ID NO: 120 - protein, 452 aa, Artificial Sequence
  N/A
EVQLVQSGAEVKKPGASVKVSCKTSGYTFTEYIMHWVRQAPGQGLEWMGGIIPNNGGTSYNQKFQGRVTMTVDKSTSTGYMELSSLRSEDTAVYYCTRREVYGRNYYALDYWGQGTLVTVSSASTKGPSVFPLAPSSKSTSGGTAALGCLVKDYFPEPVTVSWNSGALTSGVHTFPAVLQSSGLYSLSSVVTVPSSSLGTQTYICNVNHKPSNTKVDKRVEPKSCDKTHTCPPCPAPEFEGGPSVFLFPPKPKDTLMISRTPEVTCVVVAVSHEDPEVKFNWYVDGVEVHNAKTKPREEQYNSTYRVVSVLTVLHQDWLNGKEYKCKVSNKALPAPIEKTISKAKGQPREPQVYTLPPSREEMTKNQVSLTCLVKGFYPSDIAVEWESNGQPENNYKTTPPVLDSDGSFFLYSRLTVDKSRWQQGNVFSCSVMHEALHNHYTQKSLSLSPGK

SEQ ID NO: 121 - protein, 107 aa, Artificial Sequence
  N/A
DIQMTQSPSSLSASVGDRVTITCSASQGINNYLNWYQQKPGKAVKLLIYYTSSLHSGVPSRFSGSGSGTDYTFTISSLQPEDIATYYCQQYSNLPYTFGGGTKVEIK

SEQ ID NO: 122 - protein, 214 aa, Artificial Sequence
  N/A
DIQMTQSPSSLSASVGDRVTITCSASQGINNYLNWYQQKPGKAVKLLIYYTSSLHSGVPSRFSGSGSGTDYTFTISSLQPEDIATYYCQQYSNLPYTFGGGTKVEIKRTVAAPSVFIFPPSDEQLKSGTASVVCLLNNFYPREAKVQWKVDNALQSGNSQESVTEQDSKDSTYSLSSTLTLSKADYEKHKVYACEVTHQGLSSPVTKSFNRGEC

SEQ ID NO: 123 - protein, 117 aa, Artificial Sequence
  N/A
EVQLVESGGGLVQPGRSLRLSCTASGFSLNDYWMSWVRQAPGKGLEWVGYIDVGGSLYYAASVKGRFTISRDDSKSIAYLQMNSLKTEDTAVYYCARGGLTYGFDLWGQGTLVTVSS

SEQ ID NO: 124 - protein, 447 aa, Artificial Sequence
  N/A
EVQLVESGGGLVQPGRSLRLSCTASGFSLNDYWMSWVRQAPGKGLEWVGYIDVGGSLYYAASVKGRFTISRDDSKSIAYLQMNSLKTEDTAVYYCARGGLTYGFDLWGQGTLVTVSSASTKGPSVFPLAPSSKSTSGGTAALGCLVKDYFPEPVTVSWNSGALTSGVHTFPAVLQSSGLYSLSSVVTVPSSSLGTQTYICNVNHKPSNTKVDKRVEPKSCDKTHTCPPCPAPELLGGPSVFLFPPKPKDTLMISRTPEVTCVVVDVSHEDPEVKFNWYVDGVEVHNAKTKPREEQYNSTYRVVSVLTVLHQDWLNGKEYKCKVSNKALPAPIEKTISKAKGQPREPQVYTLPPSREEMTKNQVSLTCLVKGFYPSDIAVEWESNGQPENNYKTTPPVLDSDGSFFLYSKLTVDKSRWQQGNVFSCSVMHEALHNHYTQKSLSLSPGK

SEQ ID NO: 125 - protein, 447 aa, Artificial Sequence
  N/A
EVQLVESGGGLVQPGRSLRLSCTASGFSLNDYWMSWVRQAPGKGLEWVGYIDVGGSLYYAASVKGRFTISRDDSKSIAYLQMNSLKTEDTAVYYCARGGLTYGFDLWGQGTLVTVSSASTKGPSVFPLAPSSKSTSGGTAALGCLVKDYFPEPVTVSWNSGALTSGVHTFPAVLQSSGLYSLSSVVTVPSSSLGTQTYICNVNHKPSNTKVDKRVEPKSCDKTHTCPPCPAPEFEGGPSVFLFPPKPKDTLMISRTPEVTCVVVAVSHEDPEVKFNWYVDGVEVHNAKTKPREEQYNSTYRVVSVLTVLHQDWLNGKEYKCKVSNKALPAPIEKTISKAKGQPREPQVYTLPPSREEMTKNQVSLTCLVKGFYPSDIAVEWESNGQPENNYKTTPPVLDSDGSFFLYSRLTVDKSRWQQGNVFSCSVMHEALHNHYTQKSLSLSPGK

SEQ ID NO: 126 - protein, 447 aa, Artificial Sequence
  N/A
EVQLVESGGGLVQPGRSLRLSCTASGFSLNDYWMSWVRQAPGKGLEWVGYIDVGGSLYYAASVKGRFTISRDDSKSIAYLQMNSLKTEDTAVYYCARGGLTYGFDLWGQGTLVTVSSASTKGPSVFPLAPSSKSTSGGTAALGCLVKDYFPEPVTVSWNSGALTSGVHTFPAVLQSSGLYSLSSVVTVPSSSLGTQTYICNVNHKPSNTKVDKRVEPKSCDKTHTCPPCPAPEFEGGPSVFLFPPKPKDTLMISRTPEVTCVVVAVSHEDPEVKFNWYVDGVEVHNAKTKPREEQYNSTYRVVSVLTVLHQDWLNGKEYKCKVSNKALPAPIEKTISKAKGQPREPQVYTLPPSREEMTKNQVSLTCLVKGFYPSDIAVEWESNGQPENNYKTTPPVLDSDGSFLLYSKLTVDKSRWQQGNVFSCSVMHEALHNHYTQKSLSLSPGK

SEQ ID NO: 127 - protein, 110 aa, Artificial Sequence
  N/A
DIVMTQSPSSLSASVGDRVTITCQASEDISSYLAWYQQKPGKAPKRLIYGASDLASGVPSRFSASGSGTDYTFTISSLQPEDIATYYCHYYATISGLGVAFGGGTKVEIK

SEQ ID NO: 128 - protein, 217 aa, Artificial Sequence
  N/A
DIVMTQSPSSLSASVGDRVTITCQASEDISSYLAWYQQKPGKAPKRLIYGASDLASGVPSRFSASGSGTDYTFTISSLQPEDIATYYCHYYATISGLGVAFGGGTKVEIKRTVAAPSVFIFPPSDEQLKSGTASVVCLLNNFYPREAKVQWKVDNALQSGNSQESVTEQDSKDSTYSLSSTLTLSKADYEKHKVYACEVTHQGLSSPVTKSFNRGEC

SEQ ID NO: 129 - protein, 24 aa, Homo Sapiens
LQDPCSNCPAGTFCDNNRNQICSP

SEQ ID NO: 130 - protein, 41 aa, Homo Sapiens
CPPNSFSSAGGQRTCDICRQCKGVFRTRKECSSTSNAECDC

SEQ ID NO: 131 - protein, 26 aa, Homo Sapiens
TPGFHCLGAGCSMCEQDCKQGQELTK

SEQ ID NO: 132 - protein, 24 aa, Homo Sapiens
KGCKDCCFGTFNDQKRGICRPWTN

SEQ ID NO: 133 - protein, 23 aa, Homo Sapiens
CSLDGKSVLVNGTKERDVVCGPS

SEQ ID NO: 134 - protein, 25 aa, Homo Sapiens
PADLSPGASSVTPPAPAREPGHSPQ

SEQ ID NO: 135 - protein, 255 aa, sus scrofa
MGNGYYNIVATVLLVMNFERTRSVPDPCSNCSAGTFCGKNIQELCMPCPSNSFSSTSGQKACNVCRKCEGVFRTKKECSSTSNAVCECVPGFRCLGAGCAMCEEYCQQGQELTQEGCKDCSFGTFNDEEHGVCRPWTDCSLAGKPVLMNGTKARDVVCGPRPTDFSPGTPSTTMPVPGGEPGHTSHVIIFFLALMSTAVFVLVSYLALRFSVVQQGRKKLLYIVKQPFLKPAQTVQEEDACSCRFPEEEEGECEL

SEQ ID NO: 136 - protein, 255 aa, loxodonta africana
MGNGYYNMVATVLLVMNFERTGAVQDSCRDCLAGTYCVKNESQICSPCPLNSFSSTGGQMNCDMCRKCEGVFKTKRACSPTRDAECECVSGFHCLGAGCTMCQQDCKQGQELTKEGCKDCCLGTFNDQKNGICRPWTNCSLEGKSVLANGTKKRDVVCGPPAADSFPDTSSVTVPAPERKPDHHPQIITFFLALISAALLFLVFFLVVRFSVAKWGRKKLLYIFKQPFIKPVQTAQEEDGCSCRFPEEEEGDCEL